European Patent Application EP 4 534 676 A1, published April 9, 2025. Title: CHIMERIC ANTIGEN RECEPTOR-EXPRESSING CELLS TARGETING EGFR. Applicant: SHINSHU UNIVERSITY. The sequence listing filed with the application follows.

SEQUENCE LISTING (20 sequences)

SEQ ID NO: 1 - DNA, 159 bp, synthetic construct
  misc_feature 1..159: note = synthetic
  source 1..159: mol_type = other DNA
aatagtgactctgaatgtcccctgtcccacgatgggtactgcctccatgatggtgtgtgcatgtatattgaagcattggacaagtatgcatgcaactgtgttgttggctacatcggggagcgatgtcagtaccgagacctgaagtggtgggaactgcgc

SEQ ID NO: 2 - protein, 53 aa, Homo sapiens
NSDSECPLSHDGYCLHDGVCMYIEALDKYACNCVVGYIGERCQYRDLKWWELR

SEQ ID NO: 3 - DNA, 150 bp, synthetic construct
  misc_feature 1..150: note = synthetic
  source 1..150: mol_type = other DNA
gtggtgtcccattttaatgactgcccagattcccacactcagttctgcttccatggaacctgcaggtttttggtgcaggaggacaagccagcatgtgtctgccattctgggtacgttggtgcacgctgtgagcatgcggacctcctggcc

SEQ ID NO: 4 - protein, 50 aa, Homo sapiens
VVSHFNDCPDSHTQFCFHGTCRFLVQEDKPACVCHSGYVGARCEHADLLA

SEQ ID NO: 5 - protein, 29 aa, synthetic construct
  REGION 1..29: note = Hinge-Spacer-Hinge
EPKSCDKTHTCPPCDPAEPKSPDKTHTCP

SEQ ID NO: 6 - protein, 113 aa, Homo sapiens
PCPAPELLGGPSVFLFPPKPKDTLMISRTPEVTCVVVDVSHEDPEVKFNWYVDGVEVHNAKTKPREEQYNSTYRVVSVLTVLHQDWLNGKEYKCKVSNKALPAPIEKTISKAK

SEQ ID NO: 7 - protein, 107 aa, Homo sapiens
GQPREPQVYTLPPSRDELTKNQVSLTCLVKGFYPSDIAVEWESNGQPENNYKTTPPVLDSDGSFFLYSKLTVDKSRWQQGNVFSCSVMHEALHNHYTQKSLSLSPGK

SEQ ID NO: 8 - protein, 68 aa, Homo sapiens
FWVLVVVGGVLACYSLLVTVAFIIFWVRSKRSRLLHSDYMNMTPRRPGPTRKHYQPYAPPRDFAAYRS

SEQ ID NO: 9 - protein, 112 aa, Homo sapiens
RVKFSRSADAPAYQQGQNQLYNELNLGRREEYDVLDKRRGRDPEMGGKPRRKNPQEGLYNELQKDKMAEAYSEIGMKGERRRGKGHDGLYQGLSTATKDTYDALHMQALPPR

SEQ ID NO: 10 - DNA, 5823 bp, synthetic construct
  misc_feature 1..5823: note = synthetic
  source 1..5823: mol_type = other DNA
ttaaccctagaaagatagtctgcgtaaaattgacgcatgcattcttgaaatattgctctctctttctaaatagcgcgaatccgtcgctgtgcatttaggacatctcagtcgccgcttggagctcccgtgaggcgtgcttgtcaatgcggtaagtgtcactgattttgaactataacgaccgcgtgagtcaaaatgacgcatgattatcttttacgtgacttttaagatttaactcatacgataattatattgttatttcatgttctacttacgtgataacttattatatatatattttcttgttatagataagatcttcaatattggccattagccatattattcattggttatatagcataaatcaatattggctattggccattgcatacgttgtatctatatcataatatgtacatttatattggctcatgtccaatatgaccgccatgttggcattgattattgactagttattaatagtaatcaattacggggtcattagttcatagcccatatatggagttccgcgttacataacttacggtaaatggcccgcctggctgaccgcccaacgacccccgcccattgacgtcaataatgacgtatgttcccatagtaacgccaatagggactttccattgacgtcaatgggtggagtatttacggtaaactgcccacttggcagtacatcaagtgtatcatatgccaagtccgccccctattgacgtcaatgacggtaaatggcccgcctggcattatgcccagtacatgaccttacgggactttcctacttggcagtacatctacgtattagtcatcgctattaccatggtgatgcggttttggcagtacaccaatgggcgtggatagcggtttgactcacggggatttccaagtctccaccccattgacgtcaatgggagtttgttttggcaccaaaatcaacgggactttccaaaatgtcgtaacaactgcgatcgcccgccccgttgacgcaaatgggcggtaggcgtgtacggtgggaggtctatataagcagagctcgtttagtgaaccgtcagatcactagaagctttattgcggtagtttatcacagttaaattgctaacgcagtcagtgcttctgacacaacagtctcgaacttaagctgcagtgactctcttaaggtagccttgcagaagttggtcgtgaggcactgggcaggtaagtatcaaggttacaagacaggtttaaggagaccaatagaaactgggcttgtcgagacagagaagactcttgcgtttctgataggcacctattggtcttactgacatccactttgcctttctctccacaggtgtccactcccagttcaattacagctcttaaggctagagtacttaatacgactcactataggctagcctcgagctcaagcttcgaattcgaatggccatggagtttgggctgagctggctttttcttgtggctattttaaaaggtgtccagtgctctagaaatagtgactctgaatgtcccctgtcccacgatgggtactgcctccatgatggtgtgtgcatgtatattgaagcattggacaagtatgcatgcaactgtgttgttggctacatcggggagcgatgtcagtaccgagacctgaagtggtgggaactgcgcgagcccaaatctcctgacaaaactcacacatgcccaccgtgcccagcacctgaactcctggggggaccgtcagtcttcctcttccccccaaaacccaaggacaccctcatgatctcccggacccctgaggtcacatgcgtggtggtggacgtgagccacgaagaccctgaggtcaagttcaactggtacgtggacggcgtggaggtgcataatgccaagacaaagccgcgggaggagcagtacaacagcacgtaccgtgtggtcagcgtcctcaccgtcctgcaccaggactggctgaatggcaaggagtacaagtgcaaggtctccaacaaagccctcccagcccccatcgagaaaaccatctccaaagccaaagggcagccccgagaaccacaggtgtacaccctgcccccatcccgggatgagctgaccaagaaccaggtcagcctgacctgcctggtcaaaggcttctatcccagcgacatcgccgtggagtgggagagcaatgggcaaccggagaacaactacaagaccacgcctcccgtgctggactccgacggctccttcttcctctacagcaagctcaccgtggacaagagcaggtggcagcaggggaacgtcttctcatgctccgtgatgcatgaggctctgcacaaccactacacgcagaagagcctctccctgtctccgggtaaaaaagatcccaaattttgggtgctggtggtggttggtggagtcctggcttgctatagcttgctagtaacagtggcctttattattttctgggtgaggagtaagaggagcaggctcctgcacagtgactacatgaacatgactccccgccgccccgggcccacccgcaagcattaccagccctatgccccaccacgcgacttcgcagcctatcgctccagagtgaagttcagcaggagcgcagacgcccccgcgtaccagcagggccagaaccagctctataacgagctcaatctaggacgaagagaggagtacgatgttttggacaagagacgtggccgggaccctgagatggggggaaagccgagaaggaagaaccctcaggaaggcctgtacaatgaactgcagaaagataagatggcggaggcctacagtgagattgggatgaaaggcgagcgccggaggggcaaggggcacgatggcctttaccagggtctcagtacagccaccaaggacacctacgacgcccttcacatgcaggccctgcctcctcgctaagcatgctagctatagttctagaggtaccggttgttaacgttagccggctacgtatactccggaatattaataggcctaggatgcatatggcggccgcttccctttagtgagggttaatgcttcgagcagacatgataagatacattgatgagtttggacaaaccacaactagaatgcagtgaaaaaaatgctttatttgtgaaatttgtgatgctattgctttatttgtaaccattataagctgcaataaacaagttaacaacaacaattgcattcattttatgtttcaggttcagggggagatgtgggaggttttttaaagcaagtaaaacctctacaaatgtggtaaaatccgataaggatcgatccgggctggcgtaatagcgaagaggcccgcaccgatcgcccttcccaacagttgcgcagcctgaatggcgaatggacgcgccctgtagcggcgcattaagcgcggcgggtgtggtggttacgcgcagcgtgaccgctacacttgccagcgccctagcgcccgctcctttcgctttcttcccttcctttctcgccacgttcgcccgatagcgataaggatccgcgtatggtgcactctcagtacaatctgctctgatgccgcatagttaagccagccccgacacccgccaacacccgctgacgcgccctgacgggcttgtctgctcccggcatccgcttacagacaagctgtgaccgtctccgggattttgttactttatagaagaaattttgagtttttgtttttttttaataaataaataaacataaataaattgtttgttgaatttattattagtatgtaagtgtaaatataataaaacttaatatctattcaaattaataaataaacctcgatatacagaccgataaaacacatgcgtcaattttacgcatgattatctttaacgtacgtcacaatatgattatctttctagggttaatccgggagctgcatgtgtcagaggttttcaccgtcatcaccgaaacgcgcgagacgaaagggcctcgtgatacgcctatttttataggttaatgtcatgataataatggtttcttagacgtcaggtggcacttttcggggaaatgtgcgcggaacccctatttgtttatttttctaaatacattcaaatatgtatccgctcatgagacaataaccctgataaatgcttcaataatattgaaaaaggaagagtatgagtattcaacatttccgtgtcgcccttattcccttttttgcggcattttgccttcctgtttttgctcacccagaaacgctggtgaaagtaaaagatgctgaagatcagttgggtgcacgagtgggttacatcgaactggatctcaacagcggtaagatccttgagagttttcgccccgaagaacgttttccaatgatgagcacttttaaagttctgctatgtggcgcggtattatcccgtattgacgccgggcaagagcaactcggtcgccgcatacactattctcagaatgacttggttgagtactcaccagtcacagaaaagcatcttacggatggcatgacagtaagagaattatgcagtgctgccataaccatgagtgataacactgcggccaacttacttctgacaacgatcggaggaccgaaggagctaaccgcttttttgcacaacatgggggatcatgtaactcgccttgatcgttgggaaccggagctgaatgaagccataccaaacgacgagcgtgacaccacgatgcctgtagcaatggcaacaacgttgcgcaaactattaactggcgaactacttactctagcttcccggcaacaattaatagactggatggaggcggataaagttgcaggaccacttctgcgctcggcccttccggctggctggtttattgctgataaatctggagccggtgagcgtgggtctcgcggtatcattgcagcactggggccagatggtaagccctcccgtatcgtagttatctacacgacggggagtcaggcaactatggatgaacgaaatagacagatcgctgagataggtgcctcactgattaagcattggtaactgtcagaccaagtttactcatatatactttagattgatttaaaacttcatttttaatttaaaaggatctaggtgaagatcctttttgataatctcatgaccaaaatcccttaacgtgagttttcgttccactgagcgtcagaccccgtagaaaagatcaaaggatcttcttgagatcctttttttctgcgcgtaatctgctgcttgcaaacaaaaaaaccaccgctaccagcggtggtttgtttgccggatcaagagctaccaactctttttccgaaggtaactggcttcagcagagcgcagataccaaatactgttcttctagtgtagccgtagttaggccaccacttcaagaactctgtagcaccgcctacatacctcgctctgctaatcctgttaccagtggctgctgccagtggcgataagtcgtgtcttaccgggttggactcaagacgatagttaccggataaggcgcagcggtcgggctgaacggggggttcgtgcacacagcccagcttggagcgaacgacctacaccgaactgagatacctacagcgtgagctatgagaaagcgccacgcttcccgaagggagaaaggcggacaggtatccggtaagcggcagggtcggaacaggagagcgcacgagggagcttccagggggaaacgcctggtatctttatagtcctgtcgggtttcgccacctctgacttgagcgtcgatttttgtgatgctcgtcaggggggcggagcctatggaaaaacgccagcaacgcggcctttttacggttcctggccttttgctggccttttgctcacatggctcgacagatct

SEQ ID NO: 11 - DNA, 5814 bp, synthetic construct
  misc_feature 1..5814: note = synthetic
  source 1..5814: mol_type = other DNA
ttaaccctagaaagatagtctgcgtaaaattgacgcatgcattcttgaaatattgctctctctttctaaatagcgcgaatccgtcgctgtgcatttaggacatctcagtcgccgcttggagctcccgtgaggcgtgcttgtcaatgcggtaagtgtcactgattttgaactataacgaccgcgtgagtcaaaatgacgcatgattatcttttacgtgacttttaagatttaactcatacgataattatattgttatttcatgttctacttacgtgataacttattatatatatattttcttgttatagataagatcttcaatattggccattagccatattattcattggttatatagcataaatcaatattggctattggccattgcatacgttgtatctatatcataatatgtacatttatattggctcatgtccaatatgaccgccatgttggcattgattattgactagttattaatagtaatcaattacggggtcattagttcatagcccatatatggagttccgcgttacataacttacggtaaatggcccgcctggctgaccgcccaacgacccccgcccattgacgtcaataatgacgtatgttcccatagtaacgccaatagggactttccattgacgtcaatgggtggagtatttacggtaaactgcccacttggcagtacatcaagtgtatcatatgccaagtccgccccctattgacgtcaatgacggtaaatggcccgcctggcattatgcccagtacatgaccttacgggactttcctacttggcagtacatctacgtattagtcatcgctattaccatggtgatgcggttttggcagtacaccaatgggcgtggatagcggtttgactcacggggatttccaagtctccaccccattgacgtcaatgggagtttgttttggcaccaaaatcaacgggactttccaaaatgtcgtaacaactgcgatcgcccgccccgttgacgcaaatgggcggtaggcgtgtacggtgggaggtctatataagcagagctcgtttagtgaaccgtcagatcactagaagctttattgcggtagtttatcacagttaaattgctaacgcagtcagtgcttctgacacaacagtctcgaacttaagctgcagtgactctcttaaggtagccttgcagaagttggtcgtgaggcactgggcaggtaagtatcaaggttacaagacaggtttaaggagaccaatagaaactgggcttgtcgagacagagaagactcttgcgtttctgataggcacctattggtcttactgacatccactttgcctttctctccacaggtgtccactcccagttcaattacagctcttaaggctagagtacttaatacgactcactataggctagcctcgagctcaagcttcgaattcgaatggccatggagtttgggctgagctggctttttcttgtggctattttaaaaggtgtccagtgctctagagtggtgtcccattttaatgactgcccagattcccacactcagttctgcttccatggaacctgcaggtttttggtgcaggaggacaagccagcatgtgtctgccattctgggtacgttggtgcacgctgtgagcatgcggacctcctggccgagcccaaatctcctgacaaaactcacacatgcccaccgtgcccagcacctgaactcctggggggaccgtcagtcttcctcttccccccaaaacccaaggacaccctcatgatctcccggacccctgaggtcacatgcgtggtggtggacgtgagccacgaagaccctgaggtcaagttcaactggtacgtggacggcgtggaggtgcataatgccaagacaaagccgcgggaggagcagtacaacagcacgtaccgtgtggtcagcgtcctcaccgtcctgcaccaggactggctgaatggcaaggagtacaagtgcaaggtctccaacaaagccctcccagcccccatcgagaaaaccatctccaaagccaaagggcagccccgagaaccacaggtgtacaccctgcccccatcccgggatgagctgaccaagaaccaggtcagcctgacctgcctggtcaaaggcttctatcccagcgacatcgccgtggagtgggagagcaatgggcaaccggagaacaactacaagaccacgcctcccgtgctggactccgacggctccttcttcctctacagcaagctcaccgtggacaagagcaggtggcagcaggggaacgtcttctcatgctccgtgatgcatgaggctctgcacaaccactacacgcagaagagcctctccctgtctccgggtaaaaaagatcccaaattttgggtgctggtggtggttggtggagtcctggcttgctatagcttgctagtaacagtggcctttattattttctgggtgaggagtaagaggagcaggctcctgcacagtgactacatgaacatgactccccgccgccccgggcccacccgcaagcattaccagccctatgccccaccacgcgacttcgcagcctatcgctccagagtgaagttcagcaggagcgcagacgcccccgcgtaccagcagggccagaaccagctctataacgagctcaatctaggacgaagagaggagtacgatgttttggacaagagacgtggccgggaccctgagatggggggaaagccgagaaggaagaaccctcaggaaggcctgtacaatgaactgcagaaagataagatggcggaggcctacagtgagattgggatgaaaggcgagcgccggaggggcaaggggcacgatggcctttaccagggtctcagtacagccaccaaggacacctacgacgcccttcacatgcaggccctgcctcctcgctaagcatgctagctatagttctagaggtaccggttgttaacgttagccggctacgtatactccggaatattaataggcctaggatgcatatggcggccgcttccctttagtgagggttaatgcttcgagcagacatgataagatacattgatgagtttggacaaaccacaactagaatgcagtgaaaaaaatgctttatttgtgaaatttgtgatgctattgctttatttgtaaccattataagctgcaataaacaagttaacaacaacaattgcattcattttatgtttcaggttcagggggagatgtgggaggttttttaaagcaagtaaaacctctacaaatgtggtaaaatccgataaggatcgatccgggctggcgtaatagcgaagaggcccgcaccgatcgcccttcccaacagttgcgcagcctgaatggcgaatggacgcgccctgtagcggcgcattaagcgcggcgggtgtggtggttacgcgcagcgtgaccgctacacttgccagcgccctagcgcccgctcctttcgctttcttcccttcctttctcgccacgttcgcccgatagcgataaggatccgcgtatggtgcactctcagtacaatctgctctgatgccgcatagttaagccagccccgacacccgccaacacccgctgacgcgccctgacgggcttgtctgctcccggcatccgcttacagacaagctgtgaccgtctccgggattttgttactttatagaagaaattttgagtttttgtttttttttaataaataaataaacataaataaattgtttgttgaatttattattagtatgtaagtgtaaatataataaaacttaatatctattcaaattaataaataaacctcgatatacagaccgataaaacacatgcgtcaattttacgcatgattatctttaacgtacgtcacaatatgattatctttctagggttaatccgggagctgcatgtgtcagaggttttcaccgtcatcaccgaaacgcgcgagacgaaagggcctcgtgatacgcctatttttataggttaatgtcatgataataatggtttcttagacgtcaggtggcacttttcggggaaatgtgcgcggaacccctatttgtttatttttctaaatacattcaaatatgtatccgctcatgagacaataaccctgataaatgcttcaataatattgaaaaaggaagagtatgagtattcaacatttccgtgtcgcccttattcccttttttgcggcattttgccttcctgtttttgctcacccagaaacgctggtgaaagtaaaagatgctgaagatcagttgggtgcacgagtgggttacatcgaactggatctcaacagcggtaagatccttgagagttttcgccccgaagaacgttttccaatgatgagcacttttaaagttctgctatgtggcgcggtattatcccgtattgacgccgggcaagagcaactcggtcgccgcatacactattctcagaatgacttggttgagtactcaccagtcacagaaaagcatcttacggatggcatgacagtaagagaattatgcagtgctgccataaccatgagtgataacactgcggccaacttacttctgacaacgatcggaggaccgaaggagctaaccgcttttttgcacaacatgggggatcatgtaactcgccttgatcgttgggaaccggagctgaatgaagccataccaaacgacgagcgtgacaccacgatgcctgtagcaatggcaacaacgttgcgcaaactattaactggcgaactacttactctagcttcccggcaacaattaatagactggatggaggcggataaagttgcaggaccacttctgcgctcggcccttccggctggctggtttattgctgataaatctggagccggtgagcgtgggtctcgcggtatcattgcagcactggggccagatggtaagccctcccgtatcgtagttatctacacgacggggagtcaggcaactatggatgaacgaaatagacagatcgctgagataggtgcctcactgattaagcattggtaactgtcagaccaagtttactcatatatactttagattgatttaaaacttcatttttaatttaaaaggatctaggtgaagatcctttttgataatctcatgaccaaaatcccttaacgtgagttttcgttccactgagcgtcagaccccgtagaaaagatcaaaggatcttcttgagatcctttttttctgcgcgtaatctgctgcttgcaaacaaaaaaaccaccgctaccagcggtggtttgtttgccggatcaagagctaccaactctttttccgaaggtaactggcttcagcagagcgcagataccaaatactgttcttctagtgtagccgtagttaggccaccacttcaagaactctgtagcaccgcctacatacctcgctctgctaatcctgttaccagtggctgctgccagtggcgataagtcgtgtcttaccgggttggactcaagacgatagttaccggataaggcgcagcggtcgggctgaacggggggttcgtgcacacagcccagcttggagcgaacgacctacaccgaactgagatacctacagcgtgagctatgagaaagcgccacgcttcccgaagggagaaaggcggacaggtatccggtaagcggcagggtcggaacaggagagcgcacgagggagcttccagggggaaacgcctggtatctttatagtcctgtcgggtttcgccacctctgacttgagcgtcgatttttgtgatgctcgtcaggggggcggagcctatggaaaaacgccagcaacgcggcctttttacggttcctggccttttgctggccttttgctcacatggctcgacagatct

SEQ ID NO: 12 - DNA, 5793 bp, synthetic construct
  misc_feature 1..5793: note = synthetic
  source 1..5793: mol_type = other DNA
ttaaccctagaaagatagtctgcgtaaaattgacgcatgcattcttgaaatattgctctctctttctaaatagcgcgaatccgtcgctgtgcatttaggacatctcagtcgccgcttggagctcccgtgaggcgtgcttgtcaatgcggtaagtgtcactgattttgaactataacgaccgcgtgagtcaaaatgacgcatgattatcttttacgtgacttttaagatttaactcatacgataattatattgttatttcatgttctacttacgtgataacttattatatatatattttcttgttatagataagatcttcaatattggccattagccatattattcattggttatatagcataaatcaatattggctattggccattgcatacgttgtatctatatcataatatgtacatttatattggctcatgtccaatatgaccgccatgttggcattgattattgactagttattaatagtaatcaattacggggtcattagttcatagcccatatatggagttccgcgttacataacttacggtaaatggcccgcctggctgaccgcccaacgacccccgcccattgacgtcaataatgacgtatgttcccatagtaacgccaatagggactttccattgacgtcaatgggtggagtatttacggtaaactgcccacttggcagtacatcaagtgtatcatatgccaagtccgccccctattgacgtcaatgacggtaaatggcccgcctggcattatgcccagtacatgaccttacgggactttcctacttggcagtacatctacgtattagtcatcgctattaccatggtgatgcggttttggcagtacaccaatgggcgtggatagcggtttgactcacggggatttccaagtctccaccccattgacgtcaatgggagtttgttttggcaccaaaatcaacgggactttccaaaatgtcgtaacaactgcgatcgcccgccccgttgacgcaaatgggcggtaggcgtgtacggtgggaggtctatataagcagagctcgtttagtgaaccgtcagatcactagaagctttattgcggtagtttatcacagttaaattgctaacgcagtcagtgcttctgacacaacagtctcgaacttaagctgcagtgactctcttaaggtagccttgcagaagttggtcgtgaggcactgggcaggtaagtatcaaggttacaagacaggtttaaggagaccaatagaaactgggcttgtcgagacagagaagactcttgcgtttctgataggcacctattggtcttactgacatccactttgcctttctctccacaggtgtccactcccagttcaattacagctcttaaggctagagtacttaatacgactcactataggctagcctcgagctcaagcttcgaattcaccatgcttctcctggtgacaagccttctgctctgtgagttaccacacccagcattcctcctgatcccagacatccagatgacacagactacatcctccctgtctgcctctctgggagacagagtcaccatcagttgcagggcaagtcaggacattagtaaatatttaaattggtatcagcagaaaccagatggaactgttaaactcctgatctaccatacatcaagattacactcaggagtcccatcaaggttcagtggcagtgggtctggaacagattattctctcaccattagcaacctggagcaagaagatattgccacttacttttgccaacagggtaatacgcttccgtacacgttcggaggggggactaagttggaaataacaggctccacctctggatccggcaagcccggatctggcgagggatccaccaagggcgaggtgaaactgcaggagtcaggacctggcctggtggcgccctcacagagcctgtccgtcacatgcactgtctcaggggtctcattacccgactatggtgtaagctggattcgccagcctccacgaaagggtctggagtggctgggagtaatatggggtagtgaaaccacatactataattcagctctcaaatccagactgaccatcatcaaggacaactccaagagccaagttttcttaaaaatgaacagtctgcaaactgatgacacagccatttactactgtgccaaacattattactacggtggtagctatgctatggactactggggtcaaggaacctcagtcaccgtctcctcagcggccgcaattgaagttatgtatcctcctccttacctagacaatgagaagagcaatggaaccattatccatgtgaaagggaaacacctttgtccaagtcccctatttcccggaccttctaagcccttttgggtgctggtggtggttgggggagtcctggcttgctatagcttgctagtaacagtggcctttattattttctgggtgaggagtaagaggagcaggctcctgcacagtgactacatgaacatgactccccgccgccccgggcccacccgcaagcattaccagccctatgccccaccacgcgacttcgcagcctatcgctccagagtgaagttcagcaggagcgcagacgcccccgcgtaccagcagggccagaaccagctctataacgagctcaatctaggacgaagagaggagtacgatgttttggacaagagacgtggccgggaccctgagatggggggaaagccgagaaggaagaaccctcaggaaggcctgtacaatgaactgcagaaagataagatggcggaggcctacagtgagattgggatgaaaggcgagcgccggaggggcaaggggcacgatggcctttaccagggtctcagtacagccaccaaggacacctacgacgcccttcacatgcaggccctgccccctcgctaaggtaccggttgttaacgttagccggctacgtatactccggaatattaataggcctaggatgcatatggcggccgcttccctttagtgagggttaatgcttcgagcagacatgataagatacattgatgagtttggacaaaccacaactagaatgcagtgaaaaaaatgctttatttgtgaaatttgtgatgctattgctttatttgtaaccattataagctgcaataaacaagttaacaacaacaattgcattcattttatgtttcaggttcagggggagatgtgggaggttttttaaagcaagtaaaacctctacaaatgtggtaaaatccgataaggatcgatccgggctggcgtaatagcgaagaggcccgcaccgatcgcccttcccaacagttgcgcagcctgaatggcgaatggacgcgccctgtagcggcgcattaagcgcggcgggtgtggtggttacgcgcagcgtgaccgctacacttgccagcgccctagcgcccgctcctttcgctttcttcccttcctttctcgccacgttcgcccgatagcgataaggatccgcgtatggtgcactctcagtacaatctgctctgatgccgcatagttaagccagccccgacacccgccaacacccgctgacgcgccctgacgggcttgtctgctcccggcatccgcttacagacaagctgtgaccgtctccgggattttgttactttatagaagaaattttgagtttttgtttttttttaataaataaataaacataaataaattgtttgttgaatttattattagtatgtaagtgtaaatataataaaacttaatatctattcaaattaataaataaacctcgatatacagaccgataaaacacatgcgtcaattttacgcatgattatctttaacgtacgtcacaatatgattatctttctagggttaatccgggagctgcatgtgtcagaggttttcaccgtcatcaccgaaacgcgcgagacgaaagggcctcgtgatacgcctatttttataggttaatgtcatgataataatggtttcttagacgtcaggtggcacttttcggggaaatgtgcgcggaacccctatttgtttatttttctaaatacattcaaatatgtatccgctcatgagacaataaccctgataaatgcttcaataatattgaaaaaggaagagtatgagtattcaacatttccgtgtcgcccttattcccttttttgcggcattttgccttcctgtttttgctcacccagaaacgctggtgaaagtaaaagatgctgaagatcagttgggtgcacgagtgggttacatcgaactggatctcaacagcggtaagatccttgagagttttcgccccgaagaacgttttccaatgatgagcacttttaaagttctgctatgtggcgcggtattatcccgtattgacgccgggcaagagcaactcggtcgccgcatacactattctcagaatgacttggttgagtactcaccagtcacagaaaagcatcttacggatggcatgacagtaagagaattatgcagtgctgccataaccatgagtgataacactgcggccaacttacttctgacaacgatcggaggaccgaaggagctaaccgcttttttgcacaacatgggggatcatgtaactcgccttgatcgttgggaaccggagctgaatgaagccataccaaacgacgagcgtgacaccacgatgcctgtagcaatggcaacaacgttgcgcaaactattaactggcgaactacttactctagcttcccggcaacaattaatagactggatggaggcggataaagttgcaggaccacttctgcgctcggcccttccggctggctggtttattgctgataaatctggagccggtgagcgtgggtctcgcggtatcattgcagcactggggccagatggtaagccctcccgtatcgtagttatctacacgacggggagtcaggcaactatggatgaacgaaatagacagatcgctgagataggtgcctcactgattaagcattggtaactgtcagaccaagtttactcatatatactttagattgatttaaaacttcatttttaatttaaaaggatctaggtgaagatcctttttgataatctcatgaccaaaatcccttaacgtgagttttcgttccactgagcgtcagaccccgtagaaaagatcaaaggatcttcttgagatcctttttttctgcgcgtaatctgctgcttgcaaacaaaaaaaccaccgctaccagcggtggtttgtttgccggatcaagagctaccaactctttttccgaaggtaactggcttcagcagagcgcagataccaaatactgttcttctagtgtagccgtagttaggccaccacttcaagaactctgtagcaccgcctacatacctcgctctgctaatcctgttaccagtggctgctgccagtggcgataagtcgtgtcttaccgggttggactcaagacgatagttaccggataaggcgcagcggtcgggctgaacggggggttcgtgcacacagcccagcttggagcgaacgacctacaccgaactgagatacctacagcgtgagctatgagaaagcgccacgcttcccgaagggagaaaggcggacaggtatccggtaagcggcagggtcggaacaggagagcgcacgagggagcttccagggggaaacgcctggtatctttatagtcctgtcgggtttcgccacctctgacttgagcgtcgatttttgtgatgctcgtcaggggggcggagcctatggaaaaacgccagcaacgcggcctttttacggttcctggccttttgctggccttttgctcacatggctcgacagatct

SEQ ID NO: 13 - protein, 21 aa, synthetic construct
MEFGLSWLFLVAILKGVQCSR

SEQ ID NO: 14 - protein, 236 aa, synthetic construct
EPKSPDKTHTCPPCPAPELLGGPSVFLFPPKPKDTLMISRTPEVTCVVVDVSHEDPEVKFNWYVDGVEVHNAKTKPREEQYNSTYRVVSVLTVLHQDWLNGKEYKCKVSNKALPAPIEKTISKAKGQPREPQVYTLPPSRDELTKNQVSLTCLVKGFYPSDIAVEWESNGQPENNYKTTPPVLDSDGSFFLYSKLTVDKSRWQQGNVFSCSVMHEALHNHYTQKSLSLSPGKKDPK

SEQ ID NO: 15 - protein, 235 aa, synthetic construct
EPKSPDKTHTCPPCPAPPVAGPSVFLFPPKPKDTLMISRTPEVTCVVVDVSHEDPEVKFNWYVDGVEVHNAKTKPREEQYQSTYRVVSVLTVLHQDWLNGKEYKCKVSNKALPAPIEKTISKAKGQPREPQVYTLPPSRDELTKNQVSLTCLVKGFYPSDIAVEWESNGQPENNYKTTPPVLDSDGSFFLYSKLTVDKSRWQQGNVFSCSVMHEALHNHYTQKSLSLSPGKKDPK

SEQ ID NO: 16 - DNA, 5820 bp, synthetic construct
  source 1..5820: mol_type = other DNA
ttaaccctagaaagatagtctgcgtaaaattgacgcatgcattcttgaaatattgctctctctttctaaatagcgcgaatccgtcgctgtgcatttaggacatctcagtcgccgcttggagctcccgtgaggcgtgcttgtcaatgcggtaagtgtcactgattttgaactataacgaccgcgtgagtcaaaatgacgcatgattatcttttacgtgacttttaagatttaactcatacgataattatattgttatttcatgttctacttacgtgataacttattatatatatattttcttgttatagataagatcttcaatattggccattagccatattattcattggttatatagcataaatcaatattggctattggccattgcatacgttgtatctatatcataatatgtacatttatattggctcatgtccaatatgaccgccatgttggcattgattattgactagttattaatagtaatcaattacggggtcattagttcatagcccatatatggagttccgcgttacataacttacggtaaatggcccgcctggctgaccgcccaacgacccccgcccattgacgtcaataatgacgtatgttcccatagtaacgccaatagggactttccattgacgtcaatgggtggagtatttacggtaaactgcccacttggcagtacatcaagtgtatcatatgccaagtccgccccctattgacgtcaatgacggtaaatggcccgcctggcattatgcccagtacatgaccttacgggactttcctacttggcagtacatctacgtattagtcatcgctattaccatggtgatgcggttttggcagtacaccaatgggcgtggatagcggtttgactcacggggatttccaagtctccaccccattgacgtcaatgggagtttgttttggcaccaaaatcaacgggactttccaaaatgtcgtaacaactgcgatcgcccgccccgttgacgcaaatgggcggtaggcgtgtacggtgggaggtctatataagcagagctcgtttagtgaaccgtcagatcactagaagctttattgcggtagtttatcacagttaaattgctaacgcagtcagtgcttctgacacaacagtctcgaacttaagctgcagtgactctcttaaggtagccttgcagaagttggtcgtgaggcactgggcaggtaagtatcaaggttacaagacaggtttaaggagaccaatagaaactgggcttgtcgagacagagaagactcttgcgtttctgataggcacctattggtcttactgacatccactttgcctttctctccacaggtgtccactcccagttcaattacagctcttaaggctagagtacttaatacgactcactataggctagcctcgagctcaagcttcgaattcgaatggccatggagtttgggctgagctggctttttcttgtggctattttaaaaggtgtccagtgctctagaaatagtgactctgaatgtcccctgtcccacgatgggtactgcctccatgatggtgtgtgcatgtatattgaagcattggacaagtatgcatgcaactgtgttgttggctacatcggggagcgatgtcagtaccgagacctgaagtggtgggaactgcgcgagcccaaatctcctgacaaaactcacacatgcccaccgtgcccagcacctccagtcgcgggaccgtcagtcttcctcttccccccaaaacccaaggacaccctcatgatctcccggacccctgaggtcacatgcgtggtggtggacgtgagccacgaagaccctgaggtcaagttcaactggtacgtggacggcgtggaggtgcataatgccaagacaaagccgcgggaggagcagtaccagagcacgtaccgtgtggtcagcgtcctcaccgtcctgcaccaggactggctgaatggcaaggagtacaagtgcaaggtctccaacaaagccctcccagcccccatcgagaaaaccatctccaaagccaaagggcagccccgagaaccacaggtgtacaccctgcccccatcccgggatgagctgaccaagaaccaggtcagcctgacctgcctggtcaaaggcttctatcccagcgacatcgccgtggagtgggagagcaatgggcaaccggagaacaactacaagaccacgcctcccgtgctggactccgacggctccttcttcctctacagcaagctcaccgtggacaagagcaggtggcagcaggggaacgtcttctcatgctccgtgatgcatgaggctctgcacaaccactacacgcagaagagcctctccctgtctccgggtaaaaaagatcccaaattttgggtgctggtggtggttggtggagtcctggcttgctatagcttgctagtaacagtggcctttattattttctgggtgaggagtaagaggagcaggctcctgcacagtgactacatgaacatgactccccgccgccccgggcccacccgcaagcattaccagccctatgccccaccacgcgacttcgcagcctatcgctccagagtgaagttcagcaggagcgcagacgcccccgcgtaccagcagggccagaaccagctctataacgagctcaatctaggacgaagagaggagtacgatgttttggacaagagacgtggccgggaccctgagatggggggaaagccgagaaggaagaaccctcaggaaggcctgtacaatgaactgcagaaagataagatggcggaggcctacagtgagattgggatgaaaggcgagcgccggaggggcaaggggcacgatggcctttaccagggtctcagtacagccaccaaggacacctacgacgcccttcacatgcaggccctgcctcctcgctaagcatgctagctatagttctagaggtaccggttgttaacgttagccggctacgtatactccggaatattaataggcctaggatgcatatggcggccgcttccctttagtgagggttaatgcttcgagcagacatgataagatacattgatgagtttggacaaaccacaactagaatgcagtgaaaaaaatgctttatttgtgaaatttgtgatgctattgctttatttgtaaccattataagctgcaataaacaagttaacaacaacaattgcattcattttatgtttcaggttcagggggagatgtgggaggttttttaaagcaagtaaaacctctacaaatgtggtaaaatccgataaggatcgatccgggctggcgtaatagcgaagaggcccgcaccgatcgcccttcccaacagttgcgcagcctgaatggcgaatggacgcgccctgtagcggcgcattaagcgcggcgggtgtggtggttacgcgcagcgtgaccgctacacttgccagcgccctagcgcccgctcctttcgctttcttcccttcctttctcgccacgttcgcccgatagcgataaggatccgcgtatggtgcactctcagtacaatctgctctgatgccgcatagttaagccagccccgacacccgccaacacccgctgacgcgccctgacgggcttgtctgctcccggcatccgcttacagacaagctgtgaccgtctccgggattttgttactttatagaagaaattttgagtttttgtttttttttaataaataaataaacataaataaattgtttgttgaatttattattagtatgtaagtgtaaatataataaaacttaatatctattcaaattaataaataaacctcgatatacagaccgataaaacacatgcgtcaattttacgcatgattatctttaacgtacgtcacaatatgattatctttctagggttaatccgggagctgcatgtgtcagaggttttcaccgtcatcaccgaaacgcgcgagacgaaagggcctcgtgatacgcctatttttataggttaatgtcatgataataatggtttcttagacgtcaggtggcacttttcggggaaatgtgcgcggaacccctatttgtttatttttctaaatacattcaaatatgtatccgctcatgagacaataaccctgataaatgcttcaataatattgaaaaaggaagagtatgagtattcaacatttccgtgtcgcccttattcccttttttgcggcattttgccttcctgtttttgctcacccagaaacgctggtgaaagtaaaagatgctgaagatcagttgggtgcacgagtgggttacatcgaactggatctcaacagcggtaagatccttgagagttttcgccccgaagaacgttttccaatgatgagcacttttaaagttctgctatgtggcgcggtattatcccgtattgacgccgggcaagagcaactcggtcgccgcatacactattctcagaatgacttggttgagtactcaccagtcacagaaaagcatcttacggatggcatgacagtaagagaattatgcagtgctgccataaccatgagtgataacactgcggccaacttacttctgacaacgatcggaggaccgaaggagctaaccgcttttttgcacaacatgggggatcatgtaactcgccttgatcgttgggaaccggagctgaatgaagccataccaaacgacgagcgtgacaccacgatgcctgtagcaatggcaacaacgttgcgcaaactattaactggcgaactacttactctagcttcccggcaacaattaatagactggatggaggcggataaagttgcaggaccacttctgcgctcggcccttccggctggctggtttattgctgataaatctggagccggtgagcgtgggtctcgcggtatcattgcagcactggggccagatggtaagccctcccgtatcgtagttatctacacgacggggagtcaggcaactatggatgaacgaaatagacagatcgctgagataggtgcctcactgattaagcattggtaactgtcagaccaagtttactcatatatactttagattgatttaaaacttcatttttaatttaaaaggatctaggtgaagatcctttttgataatctcatgaccaaaatcccttaacgtgagttttcgttccactgagcgtcagaccccgtagaaaagatcaaaggatcttcttgagatcctttttttctgcgcgtaatctgctgcttgcaaacaaaaaaaccaccgctaccagcggtggtttgtttgccggatcaagagctaccaactctttttccgaaggtaactggcttcagcagagcgcagataccaaatactgttcttctagtgtagccgtagttaggccaccacttcaagaactctgtagcaccgcctacatacctcgctctgctaatcctgttaccagtggctgctgccagtggcgataagtcgtgtcttaccgggttggactcaagacgatagttaccggataaggcgcagcggtcgggctgaacggggggttcgtgcacacagcccagcttggagcgaacgacctacaccgaactgagatacctacagcgtgagctatgagaaagcgccacgcttcccgaagggagaaaggcggacaggtatccggtaagcggcagggtcggaacaggagagcgcacgagggagcttccagggggaaacgcctggtatctttatagtcctgtcgggtttcgccacctctgacttgagcgtcgatttttgtgatgctcgtcaggggggcggagcctatggaaaaacgccagcaacgcggcctttttacggttcctggccttttgctggccttttgctcacatggctcgacagatct

SEQ ID NO: 17 - DNA, 5811 bp, synthetic construct
  source 1..5811: mol_type = other DNA
ttaaccctagaaagatagtctgcgtaaaattgacgcatgcattcttgaaatattgctctctctttctaaatagcgcgaatccgtcgctgtgcatttaggacatctcagtcgccgcttggagctcccgtgaggcgtgcttgtcaatgcggtaagtgtcactgattttgaactataacgaccgcgtgagtcaaaatgacgcatgattatcttttacgtgacttttaagatttaactcatacgataattatattgttatttcatgttctacttacgtgataacttattatatatatattttcttgttatagataagatcttcaatattggccattagccatattattcattggttatatagcataaatcaatattggctattggccattgcatacgttgtatctatatcataatatgtacatttatattggctcatgtccaatatgaccgccatgttggcattgattattgactagttattaatagtaatcaattacggggtcattagttcatagcccatatatggagttccgcgttacataacttacggtaaatggcccgcctggctgaccgcccaacgacccccgcccattgacgtcaataatgacgtatgttcccatagtaacgccaatagggactttccattgacgtcaatgggtggagtatttacggtaaactgcccacttggcagtacatcaagtgtatcatatgccaagtccgccccctattgacgtcaatgacggtaaatggcccgcctggcattatgcccagtacatgaccttacgggactttcctacttggcagtacatctacgtattagtcatcgctattaccatggtgatgcggttttggcagtacaccaatgggcgtggatagcggtttgactcacggggatttccaagtctccaccccattgacgtcaatgggagtttgttttggcaccaaaatcaacgggactttccaaaatgtcgtaacaactgcgatcgcccgccccgttgacgcaaatgggcggtaggcgtgtacggtgggaggtctatataagcagagctcgtttagtgaaccgtcagatcactagaagctttattgcggtagtttatcacagttaaattgctaacgcagtcagtgcttctgacacaacagtctcgaacttaagctgcagtgactctcttaaggtagccttgcagaagttggtcgtgaggcactgggcaggtaagtatcaaggttacaagacaggtttaaggagaccaatagaaactgggcttgtcgagacagagaagactcttgcgtttctgataggcacctattggtcttactgacatccactttgcctttctctccacaggtgtccactcccagttcaattacagctcttaaggctagagtacttaatacgactcactataggctagcctcgagctcaagcttcgaattcgaatggccatggagtttgggctgagctggctttttcttgtggctattttaaaaggtgtccagtgctctagagtggtgtcccattttaatgactgcccagattcccacactcagttctgcttccatggaacctgcaggtttttggtgcaggaggacaagccagcatgtgtctgccattctgggtacgttggtgcacgctgtgagcatgcggacctcctggccgagcccaaatctcctgacaaaactcacacatgcccaccgtgcccagcacctccagtcgcgggaccgtcagtcttcctcttccccccaaaacccaaggacaccctcatgatctcccggacccctgaggtcacatgcgtggtggtggacgtgagccacgaagaccctgaggtcaagttcaactggtacgtggacggcgtggaggtgcataatgccaagacaaagccgcgggaggagcagtaccagagcacgtaccgtgtggtcagcgtcctcaccgtcctgcaccaggactggctgaatggcaaggagtacaagtgcaaggtctccaacaaagccctcccagcccccatcgagaaaaccatctccaaagccaaagggcagccccgagaaccacaggtgtacaccctgcccccatcccgggatgagctgaccaagaaccaggtcagcctgacctgcctggtcaaaggcttctatcccagcgacatcgccgtggagtgggagagcaatgggcaaccggagaacaactacaagaccacgcctcccgtgctggactccgacggctccttcttcctctacagcaagctcaccgtggacaagagcaggtggcagcaggggaacgtcttctcatgctccgtgatgcatgaggctctgcacaaccactacacgcagaagagcctctccctgtctccgggtaaaaaagatcccaaattttgggtgctggtggtggttggtggagtcctggcttgctatagcttgctagtaacagtggcctttattattttctgggtgaggagtaagaggagcaggctcctgcacagtgactacatgaacatgactccccgccgccccgggcccacccgcaagcattaccagccctatgccccaccacgcgacttcgcagcctatcgctccagagtgaagttcagcaggagcgcagacgcccccgcgtaccagcagggccagaaccagctctataacgagctcaatctaggacgaagagaggagtacgatgttttggacaagagacgtggccgggaccctgagatggggggaaagccgagaaggaagaaccctcaggaaggcctgtacaatgaactgcagaaagataagatggcggaggcctacagtgagattgggatgaaaggcgagcgccggaggggcaaggggcacgatggcctttaccagggtctcagtacagccaccaaggacacctacgacgcccttcacatgcaggccctgcctcctcgctaagcatgctagctatagttctagaggtaccggttgttaacgttagccggctacgtatactccggaatattaataggcctaggatgcatatggcggccgcttccctttagtgagggttaatgcttcgagcagacatgataagatacattgatgagtttggacaaaccacaactagaatgcagtgaaaaaaatgctttatttgtgaaatttgtgatgctattgctttatttgtaaccattataagctgcaataaacaagttaacaacaacaattgcattcattttatgtttcaggttcagggggagatgtgggaggttttttaaagcaagtaaaacctctacaaatgtggtaaaatccgataaggatcgatccgggctggcgtaatagcgaagaggcccgcaccgatcgcccttcccaacagttgcgcagcctgaatggcgaatggacgcgccctgtagcggcgcattaagcgcggcgggtgtggtggttacgcgcagcgtgaccgctacacttgccagcgccctagcgcccgctcctttcgctttcttcccttcctttctcgccacgttcgcccgatagcgataaggatccgcgtatggtgcactctcagtacaatctgctctgatgccgcatagttaagccagccccgacacccgccaacacccgctgacgcgccctgacgggcttgtctgctcccggcatccgcttacagacaagctgtgaccgtctccgggattttgttactttatagaagaaattttgagtttttgtttttttttaataaataaataaacataaataaattgtttgttgaatttattattagtatgtaagtgtaaatataataaaacttaatatctattcaaattaataaataaacctcgatatacagaccgataaaacacatgcgtcaattttacgcatgattatctttaacgtacgtcacaatatgattatctttctagggttaatccgggagctgcatgtgtcagaggttttcaccgtcatcaccgaaacgcgcgagacgaaagggcctcgtgatacgcctatttttataggttaatgtcatgataataatggtttcttagacgtcaggtggcacttttcggggaaatgtgcgcggaacccctatttgtttatttttctaaatacattcaaatatgtatccgctcatgagacaataaccctgataaatgcttcaataatattgaaaaaggaagagtatgagtattcaacatttccgtgtcgcccttattcccttttttgcggcattttgccttcctgtttttgctcacccagaaacgctggtgaaagtaaaagatgctgaagatcagttgggtgcacgagtgggttacatcgaactggatctcaacagcggtaagatccttgagagttttcgccccgaagaacgttttccaatgatgagcacttttaaagttctgctatgtggcgcggtattatcccgtattgacgccgggcaagagcaactcggtcgccgcatacactattctcagaatgacttggttgagtactcaccagtcacagaaaagcatcttacggatggcatgacagtaagagaattatgcagtgctgccataaccatgagtgataacactgcggccaacttacttctgacaacgatcggaggaccgaaggagctaaccgcttttttgcacaacatgggggatcatgtaactcgccttgatcgttgggaaccggagctgaatgaagccataccaaacgacgagcgtgacaccacgatgcctgtagcaatggcaacaacgttgcgcaaactattaactggcgaactacttactctagcttcccggcaacaattaatagactggatggaggcggataaagttgcaggaccacttctgcgctcggcccttccggctggctggtttattgctgataaatctggagccggtgagcgtgggtctcgcggtatcattgcagcactggggccagatggtaagccctcccgtatcgtagttatctacacgacggggagtcaggcaactatggatgaacgaaatagacagatcgctgagataggtgcctcactgattaagcattggtaactgtcagaccaagtttactcatatatactttagattgatttaaaacttcatttttaatttaaaaggatctaggtgaagatcctttttgataatctcatgaccaaaatcccttaacgtgagttttcgttccactgagcgtcagaccccgtagaaaagatcaaaggatcttcttgagatcctttttttctgcgcgtaatctgctgcttgcaaacaaaaaaaccaccgctaccagcggtggtttgtttgccggatcaagagctaccaactctttttccgaaggtaactggcttcagcagagcgcagataccaaatactgttcttctagtgtagccgtagttaggccaccacttcaagaactctgtagcaccgcctacatacctcgctctgctaatcctgttaccagtggctgctgccagtggcgataagtcgtgtcttaccgggttggactcaagacgatagttaccggataaggcgcagcggtcgggctgaacggggggttcgtgcacacagcccagcttggagcgaacgacctacaccgaactgagatacctacagcgtgagctatgagaaagcgccacgcttcccgaagggagaaaggcggacaggtatccggtaagcggcagggtcggaacaggagagcgcacgagggagcttccagggggaaacgcctggtatctttatagtcctgtcgggtttcgccacctctgacttgagcgtcgatttttgtgatgctcgtcaggggggcggagcctatggaaaaacgccagcaacgcggcctttttacggttcctggccttttgctggccttttgctcacatggctcgacagatct

SEQ ID NO: 18 - protein, 687 aa, synthetic construct
MRPSGTAGAALLALLAALCPASRALEEKKVCQGTSNKLTQLGTFEDHFLSLQRMFNNCEVVLGNLEITYVQRNYDLSFLKTIQEVAGYVLIALNTVERIPLENLQIIRGNMYYENSYALAVLSNYDANKTGLKELPMRNLQEILHGAVRFSNNPALCNVESIQWRDIVSSDFLSNMSMDFQNHLGSCQKCDPSCPNGSCWGAGEENCQKLTKIICAQQCSGRCRGKSPSDCCHNQCAAGCTGPRESDCLVCRKFRDEATCKDTCPPLMLYNPTTYQMDVNPEGKYSFGATCVKKCPRNYVVTDHGSCVRACGADSYEMEEDGVRKCKKCEGPCRKVCNGIGIGEFKDSLSINATNIKHFKNCTSISGDLHILPVAFRGDSFTHTPPLDPQELDILKTVKEITGFLLIQAWPENRTDLHAFENLEIIRGRTKQHGQFSLAVVSLNITSLGLRSLKEISDGDVIISGNKNLCYANTINWKKLFGTSGQKTKIISNRGENSCKATGQVCHALCSPEGCWGPEPRDCVSCRNVSRGRECVDKCNLLEGEPREFVENSECIQCHPECLPQAMNITCTGRGPDNCIQCAHYIDGPHCVKTCPAGVMGENNTLVWKYADAGHVCHLCHPNCTYGCTGPGLEGCPTNGPKIPSIATGMVGALLLLLVVALGIGLFMRRRHIVRKRTLRRLLQERE

SEQ ID NO: 19 - protein, 288 aa, synthetic construct
MGHTRRQGTSPSKCPYLNFFQLLVLAGLSHFCSGVIHVTKEVKEVATLSCGHNVSVEELAQTRIYWQKEKKMVLTMMSGDMNIWPEYKNRTIFDITNNLSIVILALRPSDEGTYECVVLKYEKDAFKREHLAEVTLSVKADFPTPSISDFEIPTSNIRRIICSTSGGFPEPHLSWLENGEELNAINTTVSQDPETELYAVSSKLDFNMTTNHSFMCLIKYGHLRVNQTFNWNTTKQEHFPDNLLPSWAITLISVNGIFVICCLTYCFAPRCRERRRNERLRRESVRPV

SEQ ID NO: 20 - protein, 254 aa, synthetic construct
MEYASDASLDPEAPWPPAPRARACRVLPWALVAGLLLLLLLAAACAVFLACPWAVSGARASPGSAASPRLREGPELSPDDPAGLLDLRQGMFAQLVAQNVLLIDGPLSWYSDPGLAGVSLTGGLSYKEDTKELVVAKAGVYYVFFQLELRRVVAGEGSGSVSLALHLQPLRSAAGAAALALTVDLPPASSEARNSAFGFQGRLLHLSAGQRLGVHLHTEARARHAWQLTQGATVLGLFRVTPEIPAGLPSPRSE